European Patent Specification EP 3 464 596 B1, published July 30, 2025. Title: THERMOSTABLE POLYMERASE INHIBITOR COMPOSITIONS AND METHODS. Applicant: Lokhov, Sergey Gall, Alexander A. Baraznenok, Vera Viazovkina, Ekaterina V. Shishkina, Irina Persing, David H. The sequence listing filed with the application follows.

SEQUENCE LISTING (111 sequences)

SEQ ID NO: 1 - DNA, 16 bp, Artificial
  Synthetic
tataattgcaaaataa

SEQ ID NO: 2 - DNA, 16 bp, Artificial
  Synthetic
ttattttgcaattata

SEQ ID NO: 3 - DNA, 12 bp, Artificial
  Synthetic
ttcttagcgttt

SEQ ID NO: 4 - DNA, 16 bp, Artificial
  Synthetic
tataattttaaaataa

SEQ ID NO: 5 - DNA, 16 bp, Artificial
  Synthetic
ttattttaaaattata

SEQ ID NO: 6 - DNA, 40 bp, Artificial
  Synthetic
  modified_base (38)..(38): n is a fluorescein dT residue
tttttttgcaggtgacaggcgcgaagcgcctgtcaccngc

SEQ ID NO: 7 - DNA, 29 bp, Artificial
  Synthetic
aaaaggcattcctgaagctgacagcattc

SEQ ID NO: 8 - DNA, 24 bp, Artificial
  Synthetic
gagagagtagcgcgagcacagcta

SEQ ID NO: 9 - DNA, 26 bp, Artificial
  Synthetic
aaaacctgccttctgcgtgagattct

SEQ ID NO: 10 - DNA, 26 bp, Artificial
  Synthetic
ctgtacgaaaagaccacagggcccat

SEQ ID NO: 11 - DNA, 16 bp, Artificial
  Synthetic
atattaaaaaattata

SEQ ID NO: 12 - DNA, 16 bp, Artificial
  Synthetic
tataattttttaatat

SEQ ID NO: 13 - DNA, 14 bp, Artificial
  Synthetic
atattaaaattata

SEQ ID NO: 14 - DNA, 14 bp, Artificial
  Synthetic
tataattttaatat

SEQ ID NO: 15 - DNA, 16 bp, Artificial
  Synthetic
atattaaaaaattata

SEQ ID NO: 16 - DNA, 16 bp, Artificial
  Synthetic
tataattttttaatat

SEQ ID NO: 17 - DNA, 16 bp, Artificial
  Synthetic
ttattttaaaattata

SEQ ID NO: 18 - DNA, 16 bp, Artificial
  Synthetic
tataattttaaaataa

SEQ ID NO: 19 - DNA, 16 bp, Artificial
  Synthetic
ttattttaaaattata

SEQ ID NO: 20 - DNA, 16 bp, Artificial
  Synthetic
tataattccaaaataa

SEQ ID NO: 21 - DNA, 16 bp, Artificial
  Synthetic
ttattttggaattata

SEQ ID NO: 22 - DNA, 16 bp, Artificial
  Synthetic
tataattgcaaaataa

SEQ ID NO: 23 - DNA, 16 bp, Artificial
  Synthetic
ttattttgcaattata

SEQ ID NO: 24 - DNA, 16 bp, Artificial
  Synthetic
tataattcgaaaataa

SEQ ID NO: 25 - DNA, 16 bp, Artificial
  Synthetic
ttattttcgaattata

SEQ ID NO: 26 - DNA, 16 bp, Artificial
  Synthetic
ttattttaaaattata

SEQ ID NO: 27 - DNA, 16 bp, Artificial
  Synthetic
tataattttaaaataa

SEQ ID NO: 28 - DNA, 16 bp, Artificial
  Synthetic
ttattttccaattata

SEQ ID NO: 29 - DNA, 16 bp, Artificial
  Synthetic
tataattggaaaataa

SEQ ID NO: 30 - DNA, 16 bp, Artificial
  Synthetic
ttattttgcaattata

SEQ ID NO: 31 - DNA, 16 bp, Artificial
  Synthetic
tataattgcaaaataa

SEQ ID NO: 32 - DNA, 16 bp, Artificial
  Synthetic
ttattttcgaattata

SEQ ID NO: 33 - DNA, 16 bp, Artificial
  Synthetic
tataattcgaaaataa

SEQ ID NO: 34 - DNA, 14 bp, Artificial
  Synthetic
tattttaaaaatat

SEQ ID NO: 35 - DNA, 14 bp, Artificial
  Synthetic
atatttttaaaata

SEQ ID NO: 36 - DNA, 14 bp, Artificial
  Synthetic
tatttttaaaatat

SEQ ID NO: 37 - DNA, 14 bp, Artificial
  Synthetic
atattttaaaaata

SEQ ID NO: 38 - DNA, 14 bp, Artificial
  Synthetic
tattttaaaaatat

SEQ ID NO: 39 - DNA, 15 bp, Artificial
  Synthetic
  misc_feature (8)..(8): n is a DMT-ethane-diol phosphoroamidite (C-2 spacer)
atattttntaaaata

SEQ ID NO: 40 - DNA, 14 bp, Artificial
  Synthetic
tatttttaaaatat

SEQ ID NO: 41 - DNA, 15 bp, Artificial
  Synthetic
  misc_feature (8)..(8): n is a DMT-ethane-diol phosphoroamidite (C-2 spacer)
atattttnaaaaata

SEQ ID NO: 42 - DNA, 56 bp, Artificial
  Synthetic
caaaataattcttagcgtttttattttgcaattatattcttagcgttttataattg

SEQ ID NO: 43 - DNA, 56 bp, Artificial
  Synthetic
caattatattcttagcgttttataattgcaaaataattcttagcgtttttattttg

SEQ ID NO: 44 - DNA, 56 bp, Artificial
  Synthetic
taaaataattcttagcgtttttattttaaaattatattcttagcgttttataattt

SEQ ID NO: 45 - DNA, 56 bp, Artificial
  Synthetic
caaaataattcttagcgtttttattttggaattatattcttagcgttttataattc

SEQ ID NO: 46 - DNA, 56 bp, Artificial
  Synthetic
gaaaataattcttagcgtttttattttcgaattatattcttagcgttttataattc

SEQ ID NO: 47 - DNA, 56 bp, Artificial
  Synthetic
aaattatattcttagcgttttataattttaaaataattcttagcgtttttatttta

SEQ ID NO: 48 - DNA, 56 bp, Artificial
  Synthetic
caattatattcttagcgttttataattggaaaataattcttagcgtttttattttc

SEQ ID NO: 49 - DNA, 56 bp, Artificial
  Synthetic
gaattatattcttagcgttttataattcgaaaataattcttagcgtttttattttc

SEQ ID NO: 50 - DNA, 52 bp, Artificial
  Synthetic
aaaatatttcttagcgtttatatttttaaaatattcttagcgttttatttta

SEQ ID NO: 51 - DNA, 52 bp, Artificial
  Synthetic
aaaatatttcttagcgtttatattttaaaaatattcttagcgttttattttt

SEQ ID NO: 52 - DNA, 53 bp, Artificial
  Synthetic
  misc_feature (27)..(27): n is a DMT-ethane-diol phosphoroamidite (C-2 spacer)
aaaatatttcttagcgtttatattttntaaaatattcttagcgttttatttta

SEQ ID NO: 53 - DNA, 53 bp, Artificial
  Synthetic
  misc_feature (27)..(27): n is a DMT-ethane-diol phosphoroamidite (C-2 spacer)
aaaatatttcttagcgtttatattttnaaaaatattcttagcgttttattttt

SEQ ID NO: 54 - DNA, 54 bp, Artificial
  Synthetic
aaattatatcttagcgttttataattttttaatattcttagcgtttatattaaa

SEQ ID NO: 55 - DNA, 50 bp, Artificial
  Synthetic
aattatatcttagcgttttataattttaatattcttagcgtttatattaa

SEQ ID NO: 56 - DNA, 56 bp, Artificial
  Synthetic
aaattatattcttagcgttttataattttttaatatttcttagcgtttatattaaa

SEQ ID NO: 57 - DNA, 56 bp, Artificial; identical to SEQ ID NO: 47
  Synthetic

SEQ ID NO: 58 - DNA, 16 bp, Artificial
  Synthetic
ttattttaaaattata

SEQ ID NO: 59 - DNA, 16 bp, Artificial
  Synthetic
tataattttaaaataa

SEQ ID NO: 60 - DNA, 16 bp, Artificial
  Synthetic
tatttttaaaaatata

SEQ ID NO: 61 - DNA, 16 bp, Artificial
  Synthetic
tatatttttaaaaata

SEQ ID NO: 62 - DNA, 16 bp, Artificial
  Synthetic
ttaatttaaatttata

SEQ ID NO: 63 - DNA, 16 bp, Artificial
  Synthetic
tataaatttaaattaa

SEQ ID NO: 64 - DNA, 16 bp, Artificial
  Synthetic
ttaattttaaaatata

SEQ ID NO: 65 - DNA, 16 bp, Artificial
  Synthetic
tatattttaaaattaa

SEQ ID NO: 66 - DNA, 16 bp, Artificial
  Synthetic
ttatttttaaaaaata

SEQ ID NO: 67 - DNA, 16 bp, Artificial
  Synthetic
tattttttaaaaataa

SEQ ID NO: 68 - DNA, 16 bp, Artificial
  Synthetic
ttatatttaaattata

SEQ ID NO: 69 - DNA, 16 bp, Artificial
  Synthetic
tataatttaaatataa

SEQ ID NO: 70 - DNA, 14 bp, Artificial
  Synthetic
tatatttttaaaaa

SEQ ID NO: 71 - DNA, 16 bp, Artificial
  Synthetic
taatttttaaaaatat

SEQ ID NO: 72 - DNA, 15 bp, Artificial
  Synthetic
taattttaaaaaata

SEQ ID NO: 73 - DNA, 15 bp, Artificial
  Synthetic
tattttttaaaatta

SEQ ID NO: 74 - DNA, 15 bp, Artificial
  Synthetic
ttatttttaaaaaat

SEQ ID NO: 75 - DNA, 15 bp, Artificial
  Synthetic
attttttaaaaataa

SEQ ID NO: 76 - DNA, 14 bp, Artificial
  Synthetic
taattttaaaaaat

SEQ ID NO: 77 - DNA, 14 bp, Artificial
  Synthetic
attttttaaaatta

SEQ ID NO: 78 - DNA, 13 bp, Artificial
  Synthetic
taattttaaaaat

SEQ ID NO: 79 - DNA, 13 bp, Artificial
  Synthetic
atttttaaaatta

SEQ ID NO: 80 - DNA, 13 bp, Artificial
  Synthetic
caattttaaaaat

SEQ ID NO: 81 - DNA, 13 bp, Artificial
  Synthetic
atttttaaaattg

SEQ ID NO: 82 - DNA, 56 bp, Artificial
  Synthetic
gcgtttttattttaaaattatattcttagcgttttataattttaaaataattctta

SEQ ID NO: 83 - DNA, 56 bp, Artificial
  Synthetic
ttattttaaaattatattcttagcgttttataattttaaaataattcttagcgttt

SEQ ID NO: 84 - DNA, 56 bp, Artificial
  Synthetic
ttcttagcgtttttattttaaaattatattcttagcgttttataattttaaaataa

SEQ ID NO: 85 - DNA, 56 bp, Artificial
  Synthetic
gcgttttataattttaaaataattcttagcgtttttattttaaaattatattctta

SEQ ID NO: 86 - DNA, 56 bp, Artificial
  Synthetic
ttcttagcgttttataattttaaaataattcttagcgtttttattttaaaattata

SEQ ID NO: 87 - DNA, 56 bp, Artificial
  Synthetic
tataattttaaaataattcttagcgtttttattttaaaattatattcttagcgttt

SEQ ID NO: 88 - DNA, 56 bp, Artificial
  Synthetic
cgtttttattttaaaattatattcttagcgttttataattttaaaataattcttag

SEQ ID NO: 89 - DNA, 56 bp, Artificial
  Synthetic
agcgtttttattttaaaattatattcttagcgttttataattttaaaataattctt

SEQ ID NO: 90 - DNA, 56 bp, Artificial
  Synthetic
gtttttattttaaaattatattcttagcgttttataattttaaaataattcttagc

SEQ ID NO: 91 - DNA, 56 bp, Artificial
  Synthetic
tagcgtttttattttaaaattatattcttagcgttttataattttaaaataattct

SEQ ID NO: 92 - DNA, 56 bp, Artificial
  Synthetic
gcgttttatttttaaaaatatattcttagcgttttatatttttaaaaatattctta

SEQ ID NO: 93 - DNA, 56 bp, Artificial
  Synthetic
gcgtttttaatttaaatttatattcttagcgttttataaatttaaattaattctta

SEQ ID NO: 94 - DNA, 56 bp, Artificial
  Synthetic
gcgtttttaattttaaaatatattcttagcgttttatattttaaaattaattctta

SEQ ID NO: 95 - DNA, 56 bp, Artificial
  Synthetic
gcgtttttatttttaaaaaatattcttagcgttttattttttaaaaataattctta

SEQ ID NO: 96 - DNA, 56 bp, Artificial
  Synthetic
gcgtttttatatttaaattatattcttagcgttttataatttaaatataattctta

SEQ ID NO: 97 - DNA, 56 bp, Artificial
  Synthetic
cgtttttatttttaaaaaatattcttagcgttttattttttaaaaataattcttag

SEQ ID NO: 98 - DNA, 56 bp, Artificial
  Synthetic
gtttttatttttaaaaaatattcttagcgttttattttttaaaaataattcttagc

SEQ ID NO: 99 - DNA, 56 bp, Artificial
  Synthetic
cgtttatatttttaaaaattattcttagcgttttaatttttaaaaatatttcttag

SEQ ID NO: 100 - DNA, 56 bp, Artificial
  Synthetic
gtttatatttttaaaaattattcttagcgttttaatttttaaaaatatttcttagc

SEQ ID NO: 101 - DNA, 54 bp, Artificial
  Synthetic
gttttaattttaaaaaatattcttagcgttttattttttaaaattattcttagc

SEQ ID NO: 102 - DNA, 54 bp, Artificial
  Synthetic
gtttttatttttaaaaaatttcttagcgtttattttttaaaaataattcttagc

SEQ ID NO: 103 - DNA, 52 bp, Artificial
  Synthetic
gttttaattttaaaaaatttcttagcgtttattttttaaaattattcttagc

SEQ ID NO: 104 - DNA, 50 bp, Artificial
  Synthetic
gttttaattttaaaaatttcttagcgtttatttttaaaattattcttagc

SEQ ID NO: 105 - DNA, 50 bp, Artificial
  Synthetic
gtttcaattttaaaaatttcttagcgtttatttttaaaattgttcttagc

SEQ ID NO: 106 - DNA, 56 bp, Artificial; identical to SEQ ID NO: 42
  Synthetic
  misc_feature (56)..(56): g is linked to a propanediol spacer (C3)

SEQ ID NO: 107 - DNA, 56 bp, Artificial; identical to SEQ ID NO: 45
  Synthetic
  Synthetic
  misc_feature (56)..(56): c is linked to a propanediol spacer (C3)

SEQ ID NO: 108 - DNA, 56 bp, Artificial; identical to SEQ ID NO: 46
  Synthetic
  Synthetic
  misc_feature (56)..(56): c is linked to a propanediol spacer (C3)

SEQ ID NO: 109 - DNA, 56 bp, Artificial; identical to SEQ ID NO: 48
  Synthetic
  Synthetic
  misc_feature (56)..(56): c is linked to a propanediol spacer (C3)

SEQ ID NO: 110 - DNA, 56 bp, Artificial; identical to SEQ ID NO: 43
  Synthetic
  Synthetic
  misc_feature (56)..(56): g is linked to a propanediol spacer (C3)

SEQ ID NO: 111 - DNA, 56 bp, Artificial; identical to SEQ ID NO: 49
  Synthetic
  Synthetic
  misc_feature (56)..(56): c is linked to a propanediol spacer (C3)